European Patent Specification EP 2 771 355 B1, published February 8, 2023. Title: UNA CELLULA EFFETTRICE MODIFICATA PER IL TRATTAMENTO DI NEOPLASIE ESPRIMENTI IL DISIALONGANGLIOSIDE GD2. Applicant: DOMINICI, Massimo CALDRER, Sara SPANO, Maria Carlotta PAOLUCCI, Paolo. Application MO2011A000270. The sequence listing filed with the application follows.

SEQUENCE LISTING (1 sequence)

SEQ ID NO: 1 - DNA, 1612 bp, Homo sapiens
atgggctggagcctgatcctcctgttcctcgtcgctgtggctacaggtaaggggctcacagtagcaggcttgaggtctggacatatatatgggtgacaatgacatccactttgcctttctctccacaggtgtgcactcggatattgtgatgacccagtctccatcctccctggctgtgtcagcaggagagaaggtcactatgaactgcagatccagtcagagtctcctcagcagtagaacccgaaagaactacttggcttggtaccagcagaaaccagggcagtctcctaaactgctgatctactgggcatctattagggaatctggggtccctgatcgcttcacaggcagtggatctgggacagatttcactctcaccatcagcagtgtgcaggctgaagacctggcagtttattactgcaagcaatcttataatcttcggacgttcggtggaggcaccaagctggaaatcaaaggcagcactagtggtagcggcaaaccaggttccggcgaaggctcgagcaaaggtgaggtgcagctgcaggagtctggacctggcctggtggcgccctcacagagcctgtccatcacttgcactgtctctgggttttcattacccagctatggtgttcactgggttcgccagcctccaggaaagggtctggagtggctgggagtaatctgggctggtggaatcacaaattataactcggctctcatgtccagactgaccatcagcaaagacaactccaagagccaagttttcttaaaaatgaacagtcttcaaactgatgacacagccatatactactgtgccagaggcggctctgattacgacggctttgcttactggggccaagggactctggtcactgtctctaccacgacgccagcgccgcgaccaccaacaccggcgcccaccatcgcgtcgcagcccctgtccctgcgcccagaggcgtgccggccagcggcggggggcgcagtgcacacgagggggctggacttcgcctgtgatatctacatctgggcgcccttggccgggacttgtggggtccttctcctgtcactggttatcaccctttactgcaaacggggcagaaagaaactcctgtatatattcaaacaaccatttatgagaccagtacaaactactcaagaggaagatggctgtagctgccgatttccagaagaagaagaaggaggatgtgaactgagagtgaagttcagcaggagcgcagacgcccccgcgtaccagcagggccagaaccagctctataacgagctcaatctaggacgaagagaggagtacgatgttttggacaagagacgtggccgggaccctgagatggggggaaagccgagaaggaagaaccctcaggaaggcctgtacaatgaactgcagaaagataagatggcggaggcctacagtgagattgggatgaaaggcgagcgccggaggggcaaggggcacgatggcctttaccagggtctcagtacagccaccaaggacacctacgacgcccttcacatgcaggccctgccccctcgctaacagccaggggatttcaccactcaaaggccagacctgcagacgcccagattatgagacaca